European Patent Specification EP 3 512 938 B1, published August 28, 2024. Title: RECOMBINANT CARDIOMYOCYTES AND CARDIOMYOCYTE CELL LINES EXPRESSING HERG. Applicant: THE GOVERNORS OF THE UNIVERSITY OF ALBERTA. The sequence listing filed with the application follows.

SEQUENCE LISTING (2 sequences)

SEQ ID NO: 1 - protein, 1185 aa, Artificial Sequence
  Synthetic construct
MPVRRGHVAPQNTFLDTIIRKFEGQSRKFIIANARVENCAVIYCNDGFCELCGYSRAEVMQRPCTCDFLHGPRTQRRAAAQIAQALLGAEERKVEIAFYRKDGSCFLCLVDVVPVKNEDGAVIMFILNFEVVMEKDMVGSPAHDTNHRGPPTSWLAPGRAKTFRLKLPALLALTARESSVRSGGAGGAGAPGAVVVDVDLTPAAPSSESLALDEVTAMDNHVAGLGPAEERRALVGPGSPPRSAPGQLPSPRAHSLNPDASGSSCSLARTRSRESCASVRRASSADDIEAMRAGVLPPPPRHASTGAMHPLRSGLLNSTSDSDLVRYRTISKIPQITLNFVDLKGDPFLASPTSDREIIAPKIKERTHNVTEKVTQVLSLGADVLPEYKLQAPRIHRWTILHYSPFKAVWDWLILLLVIYTAVFTPYSAAFLLKETEEGPPATECGYACQPLAVVDLIVDIMFIVDILINFRTTYVNANEEVVSHPGRIAVHYFKGWFLIDMVAAIPFDLLIFGSGSEELIGLLKTARLLRLVRVARKLDRYSEYGAAVLFLLMCTFALIAHWLACIWYAIGNMEQPHMDSRIGWLHNLGDQIGKPYNSSGLGGPSIKDKYVTALYFTFSSLTSVGFGNVSPNTNSEKIFSICVMLIGSLMYASIFGNVSAIIQRLYSGTARYHTQMLRVREFIRFHQIPNPLRQRLEEYFQHAWSYTNGIDMNAVLKGFPECLQADICLHLNRSLLQHCKPFRGATKGCLRALAMKFKTTHAPPGDTLVHAGDLLTALYFISRGSIEILRGDVVVAILGKNDIFGEPLNLYARPGKSNGDVRALTYCDLHKIHRDDLLEVLDMYPEFSDHFWSSLEITFNLRDTNMIPGSPGSTELEGGFSRQRKRKLSFRRRTDKDTEQPGEVSALGPGRAGAGPSSRGRPGGPWGESPSSGPSSPESSEDEGPGRSSSPLRLVPFSSPRPPGEPPGGEPLMEDCEKSSDTCNPLSGAFSGVSNIFSFWGDSRGRQYQELPRCPAPTPSLLNIPLSSPGRRPRGDVESRLDALQRQLNRLETRLSADMATVLQLLQRQMTLVPPAYSAVTTPGPGPTSTSPLLPVSPLPTLTLDSLSQVSQFMACEELPPGAPELPQEGPTRRLSLPGQLGALTSQPLHRHGSDPGSYLECGRNPAFLYKVVLEMDYKDDDDK

SEQ ID NO: 2 - DNA, 3557 bp, Artificial Sequence
  Synthetic construct
atgccggtgcggaggggccacgtcgcgccgcagaacaccttcctggacaccatcatccgcaagtttgagggccagagccgtaagttcatcatcgccaacgctcgggtggagaactgcgccgtcatctactgcaacgacggcttctgcgagctgtgcggctactcgcgggccgaggtgatgcagcgaccctgcacctgcgacttcctgcacgggccgcgcacgcagcgccgcgctgccgcgcagatcgcgcaggcactgctgggcgccgaggagcgcaaagtggaaatcgccttctaccggaaagatgggagctgcttcctatgtctggtggatgtggtgcccgtgaagaacgaggatggggctgtcatcatgttcatcctcaatttcgaggtggtgatggagaaggacatggtggggtccccggctcatgacaccaaccaccggggcccccccaccagctggctggccccaggccgcgccaagaccttccgcctgaagctgcccgcgctgctggcgctgacggcccgggagtcgtcggtgcggtcgggcggcgcgggcggcgcgggcgccccgggggccgtggtggtggacgtggacctgacgcccgcggcacccagcagcgagtcgctggccctggacgaagtgacagccatggacaaccacgtggcagggctcgggcccgcggaggagcggcgtgcgctggtgggtcccggctctccgccccgcagcgcgcctggccagctcccatcgccccgggcgcacagcctcaaccccgacgcctcgggctccagctgcagcctggcccggacgcgctcccgagaaagctgcgccagcgtgcgccgcgcctcgtcggccgacgacatcgaggccatgcgcgccggggtgctgcccccgccaccgcgccacgccagcaccggggccatgcacccactgcgcagcggcttgctcaactccacctcggactccgacctcgtgcgctaccgcaccattagcaagattccccaaatcaccctcaactttgtggacctcaagggcgaccccttcttggcttcgcccaccagtgaccgtgagatcatagcacctaagataaaggagcgaacccacaatgtcactgagaaggtcacccaggtcctgtccctgggcgccgacgtgctgcctgagtacaagctgcaggcaccgcgcatccaccgctggaccatcctgcattacagccccttcaaggccgtgtgggactggctcatcctgctgctggtcatctacacggctgtcttcacaccctactcggctgccttcctgctgaaggagacggaagaaggcccgcctgctaccgagtgtggctacgcctgccagccgctggctgtggtggacctcatcgtggacatcatgttcattgtggacatcctcatcaacttccgcaccacctacgtcaatgccaacgaggaggtggtcagccaccccggccgcatcgccgtccactacttcaagggctggttcctcatcgacatggtggccgccatccccttcgacctgctcatcttcggctctggctctgaggagctgatcgggctgctgaagactgcgcggctgctgcggctggtgcgcgtggcgcggaagctggatcgctactcagagtacggcgcggccgtgctgttcttgctcatgtgcacctttgcgctcatcgcgcactggctagcctgcatctggtacgccatcggcaacatggagcagccacacatggactcacgcatcggctggctgcacaacctgggcgaccagataggcaaaccctacaacagcagcggcctgggcggcccctccatcaaggacaagtatgtgacggcgctctacttcaccttcagcagcctcaccagtgtgggcttcggcaacgtctctcccaacaccaactcagagaagatcttctccatctgcgtcatgctcattggctccctcatgtatgctagcatcttcggcaacgtgtcggccatcatccagcggctgtactcgggcacagcccgctaccacacacagatgctgcgggtgcgggagttcatccgcttccaccagatccccaatcccctgcgccagcgcctcgaggagtacttccagcacgcctggtcctacaccaacggcatcgacatgaacgcggtgctgaagggcttccctgagtgcctgcaggctgacatctgcctgcacctgaaccgctcactgctgcagcactgcaaacccttccgaggggccaccaagggctgccttcgggccctggccatgaagttcaagaccacacatgcaccgccaggggacacactggtgcatgctggggacctgctcaccgccctgtacttcatctcccggggctccatcgagatcctgcggggcgacgtcgtcgtggccatcctggggaagaatgacatctttggggagcctctgaacctgtatgcaaggcctggcaagtcgaacggggatgtgcgggccctcacctactgtgacctacacaagatccatcgggacgacctgctggaggtgctggacatgtaccctgagttctccgaccacttctggtccagcctggagatcaccttcaacctgcgagataccaacatgatcccgggctcccccggcagtacggagttagagggtggcttcagtcggcaacgcaagcgcaagttgtccttccgcaggcgcacggacaaggacacggagcagccaggggaggtgtcggccttggggccgggccgggcgggggcagggccgagtagccggggccggccgggggggccgtggggggagagcccgtccagtggcccctccagccctgagagcagtgaggatgagggcccaggccgcagctccagccccctccgcctggtgcccttctccagccccaggccccccggagagccgccgggtggggagcccctgatggaggactgcgagaagagcagcgacacttgcaaccccctgtcaggcgccttctcaggagtgtccaacattttcagcttctggggggacagtcggggccgccagtaccaggagctccctcgatgccccgcccccacccccagcctcctcaacatccccctctccagcccgggtcggcggccccggggcgacgtggagagcaggctggatgccctccagcgccagctcaacaggctggagacccggctgagtgcagacatggccactgtcctgcagctgctacagaggcagatgacgctggtcccgcccgcctacagtgctgtgaccaccccggggcctggccccacttccacatccccgctgttgcccgtcagccccctccccaccctcaccttggactcgctttctcaggtttcccagttcatggcgtgtgaggagctgcccccgggggccccagagcttccccaagaaggccccacacgacgcctctccctaccgggccagctgggggccctcacctcccagcccctgcacagacacggctcggacccgggcagttacctcgagtgcggccgcaacccagctttcttgtacaaagtggttctcgagatggactacaaagacgatgacgacaagta